European Patent Application EP 4 610 277 A1, published September 3, 2025. Title: METHOD FOR AVOIDING IMMUNE REJECTION USING AGONIST ON INHIBITORY KIR. Applicant: DAIICHI SANKYO COMPANY, LIMITED. Application EP 23882663.0, filed October 25, 2023. The sequence listing filed with the application follows.

SEQUENCE LISTING (146 sequences)

SEQ ID NO: 1 - protein, 21 aa, synthetic construct
  REGION 1..21: note = 2DL1 signal peptide
MSLLVVSMACVGFFLLQGAWP

SEQ ID NO: 2 - protein, 8 aa, synthetic construct
  REGION 1..8: note = flag tag
DYKDDDDK

SEQ ID NO: 3 - protein, 4 aa, synthetic construct
  REGION 1..4: note = GSGS linker
GSGS

SEQ ID NO: 4 - protein, 327 aa, synthetic construct
  REGION 1..327: note = 2DL1
HEGVHRKPSLLAHPGRLVKSEETVILQCWSDVMFEHFLLHREGMFNDTLRLIGEHHDGVSKANFSISRMTQDLAGTYRCYGSVTHSPYQVSAPSDPLDIVIIGLYEKPSLSAQLGPTVLAGENVTLSCSSRSSYDMYHLSREGEAHERRLPAGPKVNGTFQADFPLGPATHGGTYRCFGSFHDSPYEWSKSSDPLLVSVTGNPSNSWPSPTEPSSKTGNPRHLHILIGTSVVIILFILLFFLLHRWCSNKKNAAVMDQESAGNRTANSEDSDEQDPQEVTYTQLNHCVFTQRKITRPSQRPKTPPTDIIVYTELPNAESRSKVVSCP

SEQ ID NO: 5 - protein, 21 aa, synthetic construct
  REGION 1..21: note = 2DL2 signal peptide
MSLMVVSMACVGFFLLQGAWP

SEQ ID NO: 6 - protein, 327 aa, synthetic construct
  REGION 1..327: note = 2DL2
HEGVHRKPSLLAHPGRLVKSEETVILQCWSDVRFEHFLLHREGKFKDTLHLIGEHHDGVSKANFSIGPMMQDLAGTYRCYGSVTHSPYQLSAPSDPLDIVITGLYEKPSLSAQPGPTVLAGESVTLSCSSRSSYDMYHLSREGEAHECRFSAGPKVNGTFQADFPLGPATHGGTYRCFGSFRDSPYEWSNSSDPLLVSVIGNPSNSWPSPTEPSSKTGNPRHLHILIGTSVVIILFILLFFLLHRWCSNKKNAAVMDQESAGNRTANSEDSDEQDPQEVTYTQLNHCVFTQRKITRPSQRPKTPPTDIIVYAELPNAESRSKVVSCP

SEQ ID NO: 7 - protein, 21 aa, synthetic construct
  REGION 1..21: note = 2DL3 signal peptide
MSLMVVSMVCVGFFLLQGAWP

SEQ ID NO: 8 - protein, 320 aa, synthetic construct
  REGION 1..320: note = 2DL3
HEGVHRKPSLLAHPGPLVKSEETVILQCWSDVRFQHFLLHREGKFKDTLHLIGEHHDGVSKANFSIGPMMQDLAGTYRCYGSVTHSPYQLSAPSDPLDIVITGLYEKPSLSAQPGPTVLAGESVTLSCSSRSSYDMYHLSREGEAHERRFSAGPKVNGTFQADFPLGPATHGGTYRCFGSFRDSPYEWSNSSDPLLVSVTGNPSNSWPSPTEPSSETGNPRHLHVLIGTSVVIILFILLLFFLLHRWCCNKKNAVVMDQEPAGNRTVNREDSDEQDPQEVTYAQLNHCVFTQRKITRPSQRPKTPPTDIIVYTELPNAEP

SEQ ID NO: 9 - protein, 21 aa, synthetic construct
  REGION 1..21: note = 2DS1 signal peptide
MSLTVVSMACVGFFLLQGAWP

SEQ ID NO: 10 - protein, 283 aa, synthetic construct
  REGION 1..283: note = 2DS1
HEGVHRKPSLLAHPGRLVKSEETVILQCWSDVMFEHFLLHREGMFNDTLRLIGEHHDGVSKANFSISRMKQDLAGTYRCYGSVTHSPYQLSAPSDPLDIVIIGLYEKPSLSAQPGPTVLAGENVTLSCSSRSSYDMYHLSREGEAHERRLPAGTKVNGTFQANFPLGPATHGGTYRCFGSFRDSPYEWSKSSDPLLVSVTGNPSNSWPSPTEPSSETGNPRHLHVLIGTSVVKIPFTILLFFLLHRWCSDKKNAAVMDQEPAGNRTVNSEDSDEQDHQEVSYA

SEQ ID NO: 11 - protein, 21 aa, synthetic construct
  REGION 1..21: note = 2DS2 sig1nalpeptide
MSLMVVSMACVGFFLLQGAWP

SEQ ID NO: 12 - protein, 283 aa, synthetic construct
  REGION 1..283: note = 2DS2
HEGVHRKPSLLAHPGPLVKSEETVILQCWSDVRFEHFLLHREGKYKDTLHLIGEHHDGVSKANFSIGPMMQDLAGTYRCYGSVTHSPYQLSAPSDPLDIVITGLYEKPSLSAQPGPTVLAGESVTLSCSSRSSYDMYHLSREGEAHERRFSAGPKVNGTFQADFPLGPATHGGTYRCFGSFRDSPYEWSNSSDPLLVSVTGNPSNSWPSPTEPSSKTGNPRHLHVLIGTSVVKIPFTILLFFLLHRWCSNKKNAAVMDQEPAGNRTVNSEDSDEQDHQEVSYA

SEQ ID NO: 13 - protein, 21 aa, synthetic construct
  REGION 1..21: note = 2DS4 signal peptide
MSLMVIIMACVGFFLLQGAWP

SEQ ID NO: 14 - protein, 283 aa, synthetic construct
  REGION 1..283: note = 2DS4
QEGVHRKPSFLALPGHLVKSEETVILQCWSDVMFEHFLLHREGKFNNTLHLIGEHHDGVSKANFSIGPMMPVLAGTYRCYGSVPHSPYQLSAPSDPLDMVIIGLYEKPSLSAQPGPTVQAGENVTLSCSSRSSYDMYHLSREGEAHERRLPAVRSINGTFQADFPLGPATHGGTYRCFGSFRDAPYEWSNSSDPLLVSVTGNPSNSWPSPTEPSSKTGNPRHLHVLIGTSVVKIPFTILLFFLLHRWCSDKKNAAVMDQEPAGNRTVNSEDSDEQDHQEVSYA

SEQ ID NO: 15 - protein, 21 aa, synthetic construct
  REGION 1..21: note = 3DL1 signal peptide
MLLMVVSMACVGFFLVQRAGP

SEQ ID NO: 16 - protein, 423 aa, synthetic construct
  REGION 1..423: note = 3DL1
HVGGQDKPFLSAWPSAVVPRGGHVTLRCHYRHRFNNFMLYKEDRIHVPIFHGRLFQESFNMSPVTTAHAGNYTCRGSHPHSPTGWSAPSNPVVIMVTGNHRKPSLLAHPGPLVKSGERVILQCWSDIMFEHFFLHKEGISKDPSRLVGQIHDGVSKANFSIGPMMLALAGTYRCYGSVTHTPYQLSAPSDPLDIVVTGPYEKPSLSAQPGPKVQAGESVTLSCSSRSSYDMYHLSREGGAHERRLPAVRKVNRTFQADFPLGPATHGGTYRCFGSFRHSPYEWSDPSDPLLVSVTGNPSSSWPSPTEPSSKSGNPRHLHILIGTSVVIILFILLLFFLLHLWCSNKKNAAVMDQEPAGNRTANSEDSDEQDPEEVTYAQLDHCVFTQRKITRPSQRPKTPPTDTILYTELPNAKPRSKVVSCP

SEQ ID NO: 17 - protein, 550 aa, synthetic construct
  REGION 1..550: note = Firefly Luciferase
MEDAKNIKKGPAPFYPLEDGTAGEQLHKAMKRYALVPGTIAFTDAHIEVDITYAEYFEMSVRLAEAMKRYGLNTNHRIVVCSENSLQFFMPVLGALFIGVAVAPANDIYNERELLNSMGISQPTVVFVSKKGLQKILNVQKKLPIIQKIIIMDSKTDYQGFQSMYTFVTSHLPPGFNEYDFVPESFDRDKTIALIMNSSGSTGLPKGVALPHRTACVRFSHARDPIFGNQIIPDTAILSVVPFHHGFGMFTTLGYLICGFRVVLMYRFEEELFLRSLQDYKIQSALLVPTLFSFFAKSTLIDKYDLSNLHEIASGGAPLSKEVGEAVAKRFHLPGIRQGYGLTETTSAILITPEGDDKPGAVGKVVPFFEAKVVDLDTGKTLGVNQRGELCVRGPMIMSGYVNNPEATNALIDKDGWLHSGDIAYWDEDEHFFIVDRLKSLIKYKGYQVAPAELESILLQHPNIFDAGVAGLPDDDAGELPAAVVVLEHGKTMTEKEIVDYVASQVTTAKKLRGGVVFVDEVPKGLTGKLDARKIREILIKAKKGGKIAV

SEQ ID NO: 18 - protein, 20 aa, synthetic construct
  REGION 1..20: note = B2M signal peptide
MSRSVALAVLALLSLSGLEA

SEQ ID NO: 19 - protein, 99 aa, synthetic construct [sequence omitted]

SEQ ID NO: 20 - protein, 18 aa, synthetic construct
  REGION 1..18: note = T2A
EGRGSLLTCGDVEENPGP

SEQ ID NO: 21 - protein, 24 aa, synthetic construct
  REGION 1..24: note = HLA-Cw3 signal peptide
MRVMAPRTLILLLSGALALTETWA

SEQ ID NO: 22 - protein, 342 aa, synthetic construct
  REGION 1..342: note = HLA-Cw3
GSHSMRYFYTAVSRPGRGEPHFIAVGYVDDTQFVRFDSDAASPRGEPRAPWVEQEGPEYWDRETQKYKRQAQTDRVSLRNLRGYYNQSEAGSHILQRMYGCDVGPDGRLLRGYDQSAYDGKDYIALNEDLRSWTAADTAAQITQRKWEAAREAEQLRAYLEGLCVEWLRRYLKNGKETLQRAEHPKTHVTHHPVSDHEATLRCWALGFYPAEITLTWQWDGEDQTQDTELVETRPAGDGTFQKWAAVVVPSGEEQRYTCHVQHEGLPEPLTLRWEPSSQPTIPIVGIVAGLAVLAVLAVLGAVVAVVMCRRKSSGGKGGSCSQAASSNSAQGSDESLIACKA

SEQ ID NO: 23 - protein, 21 aa, synthetic construct
  REGION 1..21: note = CD8 signal peptide
MALPVTALLLPLALLLHAARP

SEQ ID NO: 24 - protein, 66 aa, synthetic construct
  REGION 1..66: note = CD8 hinge (66aa)
ALSNSIMYFSHFVPVFLPAKPTTTPAPRPPTPAPTIASQPLSLRPEACRPAAGGAVHTRGLDFACD

SEQ ID NO: 25 - protein, 15 aa, synthetic construct
  REGION 1..15: note = G4S linker
GGGGSGGGGSGGGGS

SEQ ID NO: 26 - protein, 45 aa, synthetic construct
  REGION 1..45: note = CD8 hinge (45aa)
TTTPAPRPPTPAPTIASQPLSLRPEACRPAAGGAVHTRGLDFACD

SEQ ID NO: 27 - protein, 21 aa, synthetic construct
  REGION 1..21: note = CD8 transmembrane domain
IYIWAPLAGTCGVLLLSLVIT

SEQ ID NO: 28 - protein, 5 aa, synthetic construct
  REGION 1..5: note = CD8 intracellular domain
LYCNH

SEQ ID NO: 29 - protein, 123 aa, synthetic construct
  REGION 1..123: note = Lirilumab (1-7F9) VH
QVQLVQSGAEVKKPGSSVKVSCKASGGTFSFYAISWVRQAPGQGLEWMGGFIPIFGAANYAQKFQGRVTITADESTSTAYMELSSLRSDDTAVYYCARIPSGSYYYDYDMDVWGQGTTVTVSS

SEQ ID NO: 30 - protein, 109 aa, synthetic construct
  REGION 1..109: note = Lirilumab (1-7F9) VL
EIVLTQSPVTLSLSPGERATLSCRASQSVSSYLAWYQQKPGQAPRLLIYDASNRATGIPARFSGSGSGTDFTLTISSLEPEDFAVYYCQQRSNWMYTFGQGTKLEIKRT

SEQ ID NO: 31 - protein, 121 aa, synthetic construct
  REGION 1..121: note = Pan2D VH
EVQLQQSGTVLARPGASVKMSCKASGYTFTSYWMHWMKQRPGQGLEWIGTIYPGNSDTNYNQKFKGKAKLTAVTSTNTAYMELSSLTNEDSAVYYCSRPTTATRSSAMDYWGQGTSVTVSS

SEQ ID NO: 32 - protein, 109 aa, synthetic construct
  REGION 1..109: note = Pan2D VL
QIVLTQSPASMSASLGERVTMTCTASSSVSSSYLYWYQQKPGSSPKLWIYSTSNLASGVPARFSGSGSGTSYSLTISSMEAEDAATYYCHQYHRSPPTFGGGTKLEIKR

SEQ ID NO: 33 - protein, 120 aa, synthetic construct
  REGION 1..120: note = a2DL2/3-DS1 VH
EVQLVQSGAEVKKPGSSVKVSCKASGGTFSSYAISWVRQAPGQGLEWMGGIIPIFGTANYAQKFQGRVTITADESTSTAYMELSSLRSEDTAVYYCARGELDTAIRFDYWGRGTLVTVSS

SEQ ID NO: 34 - protein, 110 aa, synthetic construct
  REGION 1..110: note = a2DL2/3-DS1 VL
QSVLTQPPSASGTPGQRVTISCSGSSSNIGSNTVNWYRQLPGTAPKLLIYSNNQRPSGVPDRFSGSKSGTSASLAISGLQSEDEADYYCAAWDDSLNGVVFGGGTKVTVL

SEQ ID NO: 35 - protein, 120 aa, synthetic construct
  REGION 1..120: note = a2DL2/3-DS2 VH
QVQLVQSGAGVKKPGSSVKVSCKASGGTFSSYAISWVRQAPGQGLEWMGGIIPIFGTSNYAQNFQGRVTITADESRNTAYMELSSLRSEDTAMYYCARGELVDPDAFDIWGQGTLVTVSS

SEQ ID NO: 36 - protein, 112 aa, synthetic construct
  REGION 1..112: note = a2DL2/3-DS2 VL
QSVLTQPPSVSGAPGQRVTISCTGSSSNIGAGYDVHWYQQLPGTAPKLLIYGNSNRPSGVPDRFSGSKSGTSASLAITGLQAEDEADYYCQSYDSSLSGYVVFGGGTKVTVL

SEQ ID NO: 37 - protein, 124 aa, synthetic construct
  REGION 1..124: note = a2DL2/3-DS3 VH
EVQLVQSGAEVKKPGSSVKVSCKASGGTFSSYAINWVRQAPGQGLEWMGGIIPIFGTANYAQKFQGRVTITADESTSTAYMELSSLRSEDTAVYYCARDHRPRGSLRGYGMDVWGQGTTVTVSS

SEQ ID NO: 38 - protein, 111 aa, synthetic construct
  REGION 1..111: note = a2DL2/3-DS3 VL
QSVVTQPPSVSGAPGQRVTISCTGSSSNIGAGYDVHWYQQLPGTAPKLLIYANNNRPSGVPDRFSGSKSGTSASLAITGLLPEDEADYYCQSYDSSLSAWVFGGGTKVTVL

SEQ ID NO: 39 - protein, 116 aa, synthetic construct
  REGION 1..116: note = a2DL2/3-DS4 VH
EVQLVQSGAEVKKPGSSVKVSCKASGGTFSSYAISWVRQAPGQGLEWMGGIIPIFGTANYAQKFQDRVTITADKSTSTAYMELSSLRSEDTAVYYCARGSRNFDYWGQGTLVTVSS

SEQ ID NO: 40 - protein, 107 aa, synthetic construct
  REGION 1..107: note = a2DL2/3-DS4 VL
AIRMTQSPSSLSASVGDRVTIPCRASQSIGSYLNWYQQKPGKAPNLLIYAASSLQSGVPSRFSGSGSGTDFTLTISSLQPEDFATYYCQQSYSTPLTFGGGTKVDIK

SEQ ID NO: 41 - protein, 121 aa, synthetic construct
  REGION 1..121: note = a2DL2/3-DS5 VH
EVQLVQSGAEVKKPGSSVKVSCKASGGTFSSYAISWVRQAPGQGLEWMGGIIPIFGTANYAQKFQGRVTMTRDTSTSTVYMELSSLRSEDTAVYYCARSKAAGTRGGMDVWGQGTLVTVSS

SEQ ID NO: 42 - protein, 107 aa, synthetic construct
  REGION 1..107: note = a2DL2/3-DS5 VL
AIRMTQSPSSLSASVGDGVTITCRASQSISSYLNWYQQKPGKAPKLLIYAASSLQSGVPSRFSGSGSGTDFTLTISSLQPEDFASYYCQQSYSTPLTFGGGTKVEIK

SEQ ID NO: 43 - protein, 124 aa, synthetic construct
  REGION 1..124: note = a2DL2/3-DS6 VH
QVQLVQSGAEVKKPGSSVKVSCKASGGTFSSYAISWVRQAPGQGLEWMGGIIPIFGTANYAQKFQGRVTITADESTSTAYMELSSLRSEDTAVYYCARGLDTPNVVVKGAFDIWGQGTTVTVSS

SEQ ID NO: 44 - protein, 108 aa, synthetic construct
  REGION 1..108: note = a2DL2/3-DS6 VL
EIVLTQSPGTLSLSPGERATLSCRASQSVSSSYLAWYQQKPGRAPRLLIYGASSRATGIPDRFSGSGSGTDFTLTISRLEPEDFAVYYCQQYGSSPWTFGQGTKLEIK

SEQ ID NO: 45 - protein, 125 aa, synthetic construct
  REGION 1..125: note = a2DL2/3-DS7 VH
EVQLVQSGAEVKKPGSSVKVSCKASGGTFSSYAISWVRQAPGQGLEWMGGIIPIFGTANYAQKFQGRVTITADESTSTAYMELSSLRSEDTAVYYCASDILTGYSVPYYYYMDVWGQGTLVTVSS

SEQ ID NO: 46 - protein, 107 aa, synthetic construct
  REGION 1..107: note = a2DL2/3-DS7 VL
DIQLTQSPSSLSASVGDRVTITCQASQDISNYLNWYQQKPGKAPKLLIYDASNLETGVPSRFSGGGSGTDFTFTISSLQPEDIATYYCQQYANLPLTFGGGTKLEIK

SEQ ID NO: 47 - protein, 122 aa, synthetic construct
  REGION 1..122: note = a2DL2/3-DS8 VH
QVQLVQSGAEVKKPGSSVKVSCKASGGTFSSYAISWVRQAPGQGLELMGGIIPIFGTANYAQKFQGRVTITADESTSTAYMELSSLRSEDTAVYYCATSGGYSYFLSPLDYWGQGTLVTVSS

SEQ ID NO: 48 - protein, 108 aa, synthetic construct
  REGION 1..108: note = a2DL2/3-DS8 VL
EIVLTQSPGTLSLSPGQRATLSCRASQSVSSNYLAWYQQKPGQAPRLLIYGASGRATGIPDRFSGSGSGTDFTLTISRLEPEDFAVYYCQQYGSSPLTFGGGTKVDIK

SEQ ID NO: 49 - protein, 122 aa, synthetic construct
  REGION 1..122: note = a2DL2/3-DS9 VH
EVQLVQSGAEVKKPGSSVKVSCKASGGTFSSYAISWVRQAPGQGLELMGGIIPIFGTANYAQKFQGRVTITADESTSTAYMELSSLRSEDTAVYYCATSGGYSYFLSPLDYWGQGTLVTVSS

SEQ ID NO: 50 - protein, 108 aa, synthetic construct; identical to SEQ ID NO: 48
  REGION 1..108: note = a2DL2/3-DS9 VL

SEQ ID NO: 51 - protein, 123 aa, synthetic construct
  REGION 1..123: note = a2DL2/3-DS10 VH
QVQLVQSGAEVKKPGSSVKVSCKASGGTFSSFAISWVRQAPGQGLEWMGGIIPIFGTANYAQKFQGRVTITADESTSTAYMELSSLRSEDTAVYYCARVSGTTGGYYYGMDVWGQGTLVTVSS

SEQ ID NO: 52 - protein, 107 aa, synthetic construct
  REGION 1..107: note = a2DL2/3-DS10 VL
AIRMTQSPSSVSASVGDRVTITCRASQGIGNWLAWYQQKPGRAPKLLISTASSLQSGVPSRFSGGGSGRGFTLTISSLQLEDFATYYCQQSYITPWTFGQGTKVEIK

SEQ ID NO: 53 - protein, 333 aa, synthetic construct
  REGION 1..333: note = Truncated CD19
MPPPRLLFFLLFLTPMEVRPEEPLVVKVEEGDNAVLQCLKGTSDGPTQQLTWSRESPLKPFLKLSLGLPGLGIHMRPLAIWLFIFNVSQQMGGFYLCQPGPPSEKAWQPGWTVNVEGSGELFRWNVSDLGGLGCGLKNRSSEGPSSPSGKLMSPKLYVWAKDRPEIWEGEPPCLPPRDSLNQSLSQDLTMAPGSTLWLSCGVPPDSVSRGPLSWTHVHPKGPKSLLSLELKDDRPARDMWVMETGLLLPRATAQDAGKYYCHRGNLTMSFHLEITARPVLWHWLLRTGGWKVSAVTLAYLIFCLCSLVGILHLQRALVLRRKRKRMTDPTRRF

SEQ ID NO: 54 - protein, 342 aa, synthetic construct
  REGION 1..342: note = HLA-Cw4
GSHSMRYFSTSVSWPGRGEPRFIAVGYVDDTQFVRFDSDAASPRGEPREPWVEQEGPEYWDRETQKYKRQAQADRVNLRKLRGYYNQSEDGSHTLQRMFGCDLGPDGRLLRGYNQFAYDGKDYIALNEDLRSWTAADTAAQITQRKWEAAREAEQRRAYLEGTCVEWLRRYLENGKETLQRAEHPKTHVTHHPVSDHEATLRCWALGFYPAEITLTWQWDGEDQTQDTELVETRPAGDGTFQKWAAVVVPSGEEQRYTCHVQHEGLPEPLTLRWKPSSQPTIPIVGIVAGLAVLAVLAVLGAMVAVVMCRRKSSGGKGGSCSQAASSNSAQGSDESLIACKA

SEQ ID NO: 55 - protein, 109 aa, synthetic construct
  REGION 1..109: note = a3DL1-DS1 VL
SYELTQPPSVSVAPGQAATITCAGDNIESKSVNWYQQKPGQAPVLVVYDDTVRPSGIPERFSGSNSGNPATLTISRSEAGDEADYYCQVWDNRRDHVVFGGGTKVTVLG

SEQ ID NO: 56 - protein, 120 aa, synthetic construct
  REGION 1..120: note = a3DL1-DS1 VH
EVQLVETGGGLVKPGGSLRLSCAASGFTFSDYYMSWIRQAPGKGLEWVSYISSSSSYTNYADSVKGRFTISRDNAKNSLYLQMNSLRAEDTAVYYCAREGIAAADAFDIWGQGTMVTVSS

SEQ ID NO: 57 - protein, 327 aa, synthetic construct
  REGION 1..327: note = KIR2DL2*003
HEGVHRKPSLLAHPGRLVKSEETVILQCWSDVRFEHFLLHREGKFKDTLHLIGEHHDGVSKANFSIGPMMQDLAGTYRCYGSVTHSPYQLSAPSDPLDIVITGLYEKPSLSAQPGPTVLAGESVTLSCSSRSSYDMYHLSREGEAHECRFSAGPKVNGTFQADFPLGPATHGGTYRCFGSFRDSPYEWSNSSDPLLVSVTGNPSNSWPSPTEPSSKTGNPRHLHILIGTSVVIILFILLFFLLHRWCSNKKNAAVMDQESAGNRTANSEDSDEQDPQEVTYTQLNHCVFTQRKITRPSQRPKTPPTDIIVYTELPNAESRSKVVSCP

SEQ ID NO: 58 - protein, 289 aa, synthetic construct
  REGION 1..289: note = Truncated NGFR
MALPVTALLLPLALLLHAARPKEACPTGLYTHSGECCKACNLGEGVAQPCGANQTVCEPCLDSVTFSDVVSATEPCKPCTECVGLQSMSAPCVEADDAVCRCAYGYYQDETTGRCEACRVCEAGSGLVFSCQDKQNTVCEECPDGTYSDEANHVDPCLPCTVCEDTERQLRECTRWADAECEEIPGRWITRSTPPEGSDSTAPSTQEPEAPPEQDLIASTVAGVVTTVMGSSQPVVTRGTTDNLIPVYCSILAAVVVGLVAYIAFKRWNSHRYPRGHRGLESTCSQAYR

SEQ ID NO: 59 - protein, 434 aa, synthetic construct
  REGION 1..434: note = KIR3DL2*002
LMGGQDKPFLSARPSTVVPRGGHVALQCHYRRGFNNFMLYKEDRSHVPIFHGRIFQESFIMGPVTPAHAGTYRCRGSRPHSLTGWSAPSNPLVIMVTGNHRKPSLLAHPGPLLKSGETVILQCWSDVMFEHFFLHRDGISEDPSRLVGQIHDGVSKANFSIGPLMPVLAGTYRCYGSVPHSPYQLSAPSDPLDIVITGLYEKPSLSAQPGPTVQAGENVTLSCSSWSSYDIYHLSREGEAHERRLRAVPKVNRTFQADFPLGPATHGGTYRCFGSFRALPCVWSNSSDPLLVSVTGNPSSSWPSPTEPSSKSGICRHLHVLIGTSVVIFLFILLLFFLLYRWCSNKKNAAVMDQEPAGDRTVNRQDSDEQDPQEVTYAQLDHCVFIQRKISRPSQRPKTPLTDTSVYTELPNAEPRSKVVSCPRAPQSGLEGVF

SEQ ID NO: 60 - protein, 361 aa, synthetic construct
  REGION 1..361: note = KIR3DS1*013
HMGGQDKPFLSAWPSAVVPRGGHVTLRCHYRHRFNNFMLYKEDRIHVPIFHGRIFQEGFNMSPVTTAHAGNYTCRGSHPHSPTGWSAPSNPMVIMVTGNHRKPSLLAHPGPLVKSGERVILQCWSDIMFEHFFLHKEWISKDPSRLVGQIHDGVSKANFSIGSMMRALAGTYRCYGSVTHTPYQLSAPSDPLDIVVTGLYEKPSLSAQPGPKVQAGESVTLSCSSRSSYDMYHLSREGGAHERRLPAVRKVNRTFQADFPLGPATHGGTYRCFGSFRHSPYEWSDPSDPLLVSVTGNPSSSWPSPTEPSSKSGNLRHLHILIGTSVVKIPFTILLFFLLHRWCSNKKKCCCNGPRACREQK

SEQ ID NO: 61 - protein, 121 aa, synthetic construct
  REGION 1..121: note = a2DL2/3-DS11 VH
QVQLVQSGAEVKKPGSSVKVSCKASGGTFSSYAISWVRQAPGQGLEWMGGIIPIFGTANYAQKFQGRVTITADESTSTAYMELSSLRSEDTAVYYCARLVSSGWYDPSDYWGQGTTVTVSS

SEQ ID NO: 62 - protein, 110 aa, synthetic construct
  REGION 1..110: note = a2DL2/3-DS11 VL
QSVLTQPPSASGTPGQRVTISCSGSSSNIGSNTVNWYQQLPGTAPKLLIYSNNQRPSGVPDRFSGSKSGTSASLAISGLQSEDEADYYCLTWDDSLTAFVFGTGTKLTVL

SEQ ID NO: 63 - protein, 121 aa, synthetic construct
  REGION 1..121: note = a2DL2/3-DS12 VH
QVQLVQSGAEVKKPGSSVKVSCKASGGTFSSYAISWVRQAPGQGLEWMGGIIPIFGTANYAQKFQGRVTITADESTSTAYMELSSLRSEDTAVYYCARVGSGWYGGDFDYWGQGTLVTVSS

SEQ ID NO: 64 - protein, 110 aa, synthetic construct
  REGION 1..110: note = a2DL2/3-DS12 VL
QSVLTQPPSVSGTPGQRVTISCSGSSSNIGSNTVNWYQQLPGTAPKLLIYTNNQRPSGVPDRFSGSKSGTSASLAISGLQSEDEADYYCAAWDDSLNGWVFGGGTKVTVL

SEQ ID NO: 65 - protein, 21 aa, synthetic construct
  REGION 1..21: note = 3DL2 signal peptide
MSLTVVSMACVGFFLLQGAWP

SEQ ID NO: 66 - protein, 21 aa, synthetic construct
  REGION 1..21: note = 3DS1 signal peptide
MLLMVVSMACVGLFLVQRAGP

SEQ ID NO: 67 - protein, 15 aa, synthetic construct
  REGION 1..15: note = R99A
AVSGTTGGYYYGMDV

SEQ ID NO: 68 - protein, 15 aa, synthetic construct
  REGION 1..15: note = V99A
RASGTTGGYYYGMDV

SEQ ID NO: 69 - protein, 15 aa, synthetic construct
  REGION 1..15: note = S100A
RVAGTTGGYYYGMDV

SEQ ID NO: 70 - protein, 15 aa, synthetic construct
  REGION 1..15: note = G101A
RVSATTGGYYYGMDV

SEQ ID NO: 71 - protein, 15 aa, synthetic construct
  REGION 1..15: note = T102A
RVSGATGGYYYGMDV

SEQ ID NO: 72 - protein, 15 aa, synthetic construct
  REGION 1..15: note = T103A
RVSGTAGGYYYGMDV

SEQ ID NO: 73 - protein, 15 aa, synthetic construct
  REGION 1..15: note = G104A
RVSGTTAGYYYGMDV

SEQ ID NO: 74 - protein, 15 aa, synthetic construct
  REGION 1..15: note = G105A
RVSGTTGAYYYGMDV

SEQ ID NO: 75 - protein, 15 aa, synthetic construct
  REGION 1..15: note = Y106A
RVSGTTGGAYYGMDV

SEQ ID NO: 76 - protein, 15 aa, synthetic construct
  REGION 1..15: note = Y107A
RVSGTTGGYAYGMDV

SEQ ID NO: 77 - protein, 15 aa, synthetic construct
  REGION 1..15: note = T108A
RVSGTTGGYYAGMDV

SEQ ID NO: 78 - protein, 15 aa, synthetic construct
  REGION 1..15: note = G109A
RVSGTTGGYYYAMDV

SEQ ID NO: 79 - protein, 15 aa, synthetic construct
  REGION 1..15: note = M110A
RVSGTTGGYYYGADV

SEQ ID NO: 80 - protein, 15 aa, synthetic construct
  REGION 1..15: note = D111A
RVSGTTGGYYYGMAV

SEQ ID NO: 81 - protein, 15 aa, synthetic construct
  REGION 1..15: note = V112A
RVSGTTGGYYYGMDA

SEQ ID NO: 82 - protein, 120 aa, synthetic construct
  REGION 1..120: note = a2DL2/3-DS1-2 VH
EVQLVQSGAEVKKPGSSVKVSCKASGGTFSSYAISWVRQAPGQGLEWMGGIIPIFGTANYAQKFQDRVTITADKSTSTAYMELSSLRSEDTAVYYCARGELDTAIRFDYWGQGTLVTVSS

SEQ ID NO: 83 - protein, 110 aa, synthetic construct
  REGION 1..110: note = a2DL2/3-DS1-2 VL
QSVLTQPPSASGTPGQRVTISCSGSSSNIGSNTVNWYQQLPGTAPKLLIYSNNQRPSGVPDRFSGSKSGTSASLAISGLRSEDEADYYCAAWDDSLNGVVFGGGTKLTVL

SEQ ID NO: 84 - protein, 120 aa, synthetic construct
  REGION 1..120: note = a2DL2/3-DS2-2 VH
EVQLVQSGAEVKKPGSSVKVSCKASGGTFSSYAISWVRQAPGQGLEWMGGIIPIFGTSNYAQKFQDRVTITADKSTSTAYMELSSLRSEDTAVYYCARGELVDPDAFDIWGQGTLVTVSS

SEQ ID NO: 85 - protein, 112 aa, synthetic construct
  REGION 1..112: note = a2DL2/3-DS2-2 VL
QSVLTQPPSASGTPGQRVTISCTGSSSNIGAGYDVHWYQQLPGTAPKLLIYGNSNRPSGVPDRFSGSKSGTSASLAISGLRSEDEADYYCQSYDSSLSGYVVFGGGTKLTVL

SEQ ID NO: 86 - protein, 124 aa, synthetic construct
  REGION 1..124: note = a2DL2/3-DS3-2 VH
EVQLVQSGAEVKKPGSSVKVSCKASGGTFSSYAINWVRQAPGQGLEWMGGIIPIFGTANYAQKFQDRVTITADKSTSTAYMELSSLRSEDTAVYYCARDHRPRGSLRGYGMDVWGQGTLVTVSS

SEQ ID NO: 87 - protein, 111 aa, synthetic construct
  REGION 1..111: note = a2DL2/3-DS3-2 VL
QSVLTQPPSASGTPGQRVTISCTGSSSNIGAGYDVHWYQQLPGTAPKLLIYANNQRPSGVPDRFSGSKSGTSASLAISGLRSEDEADYYCQSYDSSLSAWVFGGGTKLTVL

SEQ ID NO: 88 - protein, 9 aa, synthetic construct
  REGION 1..9: note = HLA-G signal peptide derived peptide
VMAPRTLFL

SEQ ID NO: 89 - protein, 20 aa, synthetic construct
  REGION 1..20: note = G4S 4 linker
GGGGSGGGGSGGGGSGGGGS

SEQ ID NO: 90 - protein, 337 aa, synthetic construct
  REGION 1..337: note = HLA-E
GSHSLKYFHTSVSRPGRGEPRFISVGYVDDTQFVRFDNDAASPRMVPRAPWMEQEGSEYWDRETRSARDTAQIFRVNLRTLRGYYNQSEAGSHTLQWMHGCELGPDRRFLRGYEQFAYDGKDYLTLNEDLRSWTAVDTAAQISEQKSNDASEAEHQRAYLEDTCVEWLHKYLEKGKETLLHLEPPKTHVTHHPISDHEATLRCWALGFYPAEITLTWQQDGEGHTQDTELVETRPAGDGTFQKWAAVVVPSGEEQRYTCHVQHEGLPEPVTLRWKPASQPTIPIVGIIAGLVLLGSVVSGAVVAAVIWRKKSSGGKGGSYSKAEWSDSAQGSESHSL

SEQ ID NO: 91 - protein, 20 aa, synthetic construct
  REGION 1..20: note = IL-2 signal peptide
MYRMQLLSCIALSLALVTNS

SEQ ID NO: 92 - protein, 6 aa, synthetic construct
  REGION 1..6: note = His tag
HHHHHH

SEQ ID NO: 93 - protein, 19 aa, synthetic construct
  REGION 1..19: note = VH signal peptide
MKHLWFFLLLVAAPRWVLS

SEQ ID NO: 94 - protein, 107 aa, synthetic construct
  REGION 1..107: note = H chain constant region of Fab fragment
ASTKGPSVFPLAPSSKSTSGGTAALGCLVKDYFPEPVTVSWNSGALTSGVHTFPAVLQSSGLYSLSSVVTVPSSSLGTQTYICNVNHKPSNTKVDKKVEPKSCDKTH

SEQ ID NO: 95 - protein, 20 aa, synthetic construct
  REGION 1..20: note = VL signal peptide
MVLQTQVFISLLLWISGAYG

SEQ ID NO: 96 - protein, 105 aa, synthetic construct [sequence omitted]

SEQ ID NO: 97 - protein, 4 aa, synthetic construct
  REGION 1..4: note = GGGS linker
GGGS

SEQ ID NO: 98 - protein, 227 aa, synthetic construct
  REGION 1..227: note = IgG Fc domain
DKTHTCPPCPAPELLGGPSVFLFPPKPKDTLMISRTPEVTCVVVDVSHEDPEVKFNWYVDGVEVHNAKTKPREEQYNSTYRVVSVLTVLHQDWLNGKEYKCKVSNKALPAPIEKTISKAKGQPREPQVYTLPPSREEMTKNQVSLTCLVKGFYPSDIAVEWESNGQPENNYKTTPPVLDSDGSFFLYSKLTVDKSRWQQGNVFSCSVMHEALHNHYTQKSLSLSPGK

SEQ ID NO: 99 - protein, 15 aa, synthetic construct
  REGION 1..15: note = Avi tag
GLNDIFEAQKIEWHE

SEQ ID NO: 100 - protein, 107 aa, synthetic construct
  REGION 1..107: note = CA19CAR VL
DIQMTQTTSSLSASLGDRVTISCRASQDISKYLNWYQQKPDGTVKLLIYHTSRLHSGVPSRFSGSGSGTDYSLTISNLEQEDIATYFCQQGNTLPYTFGGGTKLEIT

SEQ ID NO: 101 - protein, 120 aa, synthetic construct
  REGION 1..120: note = CA19CAR VH
EVKLQESGPGLVAPSQSLSVTCTVSGVSLPDYGVSWIRQPPRKGLEWLGVIWGSETTYYNSALKSRLTIIKDNSKSQVFLKMNSLQTDDTAIYYCAKHYYYGGSYAMDYWGQGTSVTVSS

SEQ ID NO: 102 - protein, 24 aa, synthetic construct
  REGION 1..24: note = CD8-derived plasma membrane domain and intracellular domain
IYIWAPLAGTCGVLLLSLVITLYC

SEQ ID NO: 103 - protein, 154 aa, synthetic construct
  REGION 1..154: note = intracellular co-stimulatory molecule
KRGRKKLLYIFKQPFMRPVQTTQEEDGCSCRFPEEEEGGCELRVKFSRSADAPAYQQGQNQLYNELNLGRREEYDVLDKRRGRDPEMGGKPRRKNPQEGLYNELQKDKMAEAYSEIGMKGERRRGKGHDGLYQGLSTATKDTYDALHMQALPPR

SEQ ID NO: 104 - protein, 233 aa, synthetic construct
  REGION 1..233: note = Blue fluorescent protein
MSELIKENMHMKLYMEGTVDNHHFKCTSEGEGKPYEGTQTMRIKVVEGGPLPFAFDILATSFLYGSKTFINHTQGIPDFFKQSFPEGFTWERVTTYEDGGVLTATQDTSLQDGCLIYNVKIRGVNFTSNGPVMQKKTLGWEAFTETLYPADGGLEGRNDMALKLVGGSHLIANIKTTYRSKKPAKNLKMPGVYYVDYRLERIKEANNETYVEQHEVAVARYCDLPSKLGHKLN

SEQ ID NO: 105 - protein, 138 aa, synthetic construct
  REGION 1..138: note = IL-21 fragment
HKSSSQGQDRHMIRMRQLIDIVDQLKNYVNDLVPEFLPAPEDVETNCEWSAFSCFQKAQLKSANTGNNERIINVSIKKLKRKPPSTNAGRRQKHRLTCPSCDSYEKKPPKEFLERFKSLLQKMIHQHLSSRTHGSEDS

SEQ ID NO: 106 - protein, 62 aa, synthetic construct
  REGION 1..62: note = CD8 hinge (62aa)
SIMYFSHFVPVFLPAKPTTTPAPRPPTPAPTIASQPLSLRPEACRPAAGGAVHTRGLDFACD

SEQ ID NO: 107 - protein, 124 aa, synthetic construct
  REGION 1..124: note = a2DL1-DS1 VH
QVQLQQSGPELVRASQTLSLTCAISGDSVSSNSATWNWIRQSPSRGLEWLGRTYYRSKWYNDYAVSVKSRITINPDTSKNQFSLQLNSVTPEDTAVYYCARDSPSYGRGVFDIWGQGTLVTVSS

SEQ ID NO: 108 - protein, 113 aa, synthetic construct
  REGION 1..113: note = a2DL1-DS1 VL
DIVMTQSPDSLAVSLGERATINCKSSQSVLYSSNNKNYLAWYQQKPGQPPKLLIYWASTRESGVPDRFSGSGSGTDFTLTISSLQAEDVAVYYCQQYYSPPYTFGQGTKLEIK

SEQ ID NO: 109 - protein, 124 aa, synthetic construct
  REGION 1..124: note = a2DL1-DS2 VH
QVQLVQSGAEVKKPGSSVKVSCKASGGTFSSYAISWVRQAPGQGLEWMGGIIPIFGTANYAQKFQGRVTITADESTSTAYMELSSLRSEDTAVYYCAREAGFWDGYNFRWFDPWGQGTLVTVSS

SEQ ID NO: 110 - protein, 107 aa, synthetic construct
  REGION 1..107: note = a2DL1-DS2 VL
EIVMTQSPATLSVSPGERATLSCRASQSVSSNLAWYQQKPGQAPRLLIYGASTRATGIPARFSGSGSGTEFTLTISSLQSEDLAIYYCQQYNNWPRTFGQGTKLEIK

SEQ ID NO: 111 - protein, 122 aa, synthetic construct
  REGION 1..122: note = a2DL1-DS3 VH
QVQLQQSGPGLVKPSQTLSLTCAISGDSVSSNSAAWNWIRQSPSRGLEWLGRTYYRSKWYNDYAVSVKSRITINPDTSKNQFSLQLNSVTPEDTAVYYCARDQTNWGLLDYWGQGTLVTVSS

SEQ ID NO: 112 - protein, 113 aa, synthetic construct
  REGION 1..113: note = a2DL1-DS3 VL
DIVMTQSPDSLAVSLGERATINCKSSQSVLYSSNNKNYLAWYQQKPGQPPKLLIYWASTRESGVPDRFSGSGSGTDFTLTISSLQAEDVAVYYCQQYYSSPWTFGQGTKVEIK

SEQ ID NO: 113 - protein, 116 aa, synthetic construct
  REGION 1..116: note = a2DL1-DS4 VH
QVQLVQSGAEVKKPGSSVKVSCKASGGTFSSYAISWVRQAPGQGLEWMGGIIPIFGTANYAQKFQGRVTITADESTSTAYMELSSLRSEDTAVYYCARSRSYFDYWGQGTLVTVSS

SEQ ID NO: 114 - protein, 108 aa, synthetic construct
  REGION 1..108: note = a2DL1-DS4 VL
EIVLTQSPGTLSLSPGEGATLSCRASQSVTSSHLAWYQQKPGQAPRLLIYGASRRATGIPDRFSGSGSGTDFTLTISRLEPEDFAVYYCQQYGSSPLTFGGGTKVEIK

SEQ ID NO: 115 - protein, 125 aa, synthetic construct
  REGION 1..125: note = a2DL1-DS5 VH
QVQLVQSGAEVKKPGASVKVSCKASGYTFTSYGISWVRQAPGQGLEWMGWISAYNGNTNYAQKLQGRVTMTTDTSTSTAYMELRSLRSDDTAVYYCALSQYYDSSGYKPDAFDIWGQGTLVTVSS

SEQ ID NO: 116 - protein, 107 aa, synthetic construct
  REGION 1..107: note = a2DL1-DS5 VL
NIQMTQSPSSLSASVGDRVTITCRASQSISSYLNWYQVKPGKAPKLLIYDASNLQSGVPSRFSGSGSGTDFTLTISSLQPEDFATYYCQQSYSTPYTFGQGTKLEIK

SEQ ID NO: 117 - protein, 117 aa, synthetic construct
  REGION 1..117: note = a2DL1-DS6 VH
QVQLVQSGAEVKKPGSSVKVSCKASGGTFSSYAISWVRQAPGQGLEWMGGIIPIFGTANYAQKFQGRVTITADESTSTAYMELSSLRSEDTAVYYCARGRSFWFDPWGQGTLVTVSS

SEQ ID NO: 118 - protein, 108 aa, synthetic construct
  REGION 1..108: note = a2DL1-DS6 VL
EIVMTQSPATLSVSPGERATLSCRASQSVSSNLAWYQQKPGQAPRLLIYGASTRATGIPARFSGSGSGTEFTLTISSLQSEDFAVYYCQQYNNWPPITFGQGTRLEIK

SEQ ID NO: 119 - protein, 123 aa, synthetic construct
  REGION 1..123: note = a2DL1-DS7 VH
EVQLLESGGGLVQPGGSLRLSCAASGFTFSSYAMHWVRQAPGKGLEWVSTISGSGGSTYYADSVKGRFAISRDNSKSTLYLRLTGLRAEDTAVYYCAKGRSRAGAGEDYFDFWGQGTLVTVSS

SEQ ID NO: 120 - protein, 110 aa, synthetic construct
  REGION 1..110: note = a2DL1-DS7 VL
QSALTQPASVSGSPGQSITISCTGTSSDVGGYNYVSWYQQHPGKAPKLMIYDVSNRPPGVSNRFSGSKSDNTASLTISGLQDEDEADYYCSSYTSSNTIIFGGGTKLTVL

SEQ ID NO: 121 - protein, 118 aa, synthetic construct
  REGION 1..118: note = a2DL1-DS8 VH
QVQLVQSGAEVKKPGSSVKVSCKASGGTFSSYAISWVRQAPGQGLEWMGGIIPIFGTANYAQKFQGRVTITADESTSTAYMELSSLRSEDTAVYYCARVYGSGSYDYWGQGTLVTVSS

SEQ ID NO: 122 - protein, 110 aa, synthetic construct
  REGION 1..110: note = a2DL1-DS8 VL
QSVVTQPPSVSAAPGQRVTISCSGSASNIGSHTVNWYQQLPGTPPKLLIYRNNQRPSGVPDRFSGSKSGTSASLAISGLQSEDEADYYCAAWDDSLNGVVFGGGTKLTVL

SEQ ID NO: 123 - protein, 117 aa, synthetic construct
  REGION 1..117: note = a2DL1-DS9 VH
QVQLVQSGAEVKKPGSSVKVSCKASGGTFSSYAISWVRQAPGQGLEWMGGIIPIFGTANYAQKFQGRVTITADESTSTAYMELSSLRSEDTAVYYCARGVRPPFPTWGQGTLVTVSS

SEQ ID NO: 124 - protein, 110 aa, synthetic construct
  REGION 1..110: note = a2DL1-DS9 VL
QSVLTQPPSASGTPGQRVTISCSGSSSNIGSNTVNWYQQFPGTAPKLLIYSNNQRPSGVPDRFSGSKSGTSASLAISGLQSEDEADYYCAAWDDSLNGWVFGGGTKLTVL

SEQ ID NO: 125 - protein, 123 aa, synthetic construct
  REGION 1..123: note = a2DL1-DS10 VH
QVQLLESGGGLVQPGGSLRLSCAASGFTFSTYATSWVRQAPGKGLEWVSTISGSGGSTYYADSVKGRFAISRDNSKSTLYLRLTGLRAEDTAVYYCAKGRSRAGAGEDYFDFWGQGTLVTVSS

SEQ ID NO: 126 - protein, 110 aa, synthetic construct
  REGION 1..110: note = a2DL1-DS10 VL
QSVLTQPPSVSAAPGQKVTISCSGGSSNIGNNYVSWYQQLPGTAPKLLIYDSNKRPSWIPDRFSGSKSGTSATLGITGLQTGDEADYYCGTWDSSLSAGVFGGGTKLTVL

SEQ ID NO: 127 - protein, 116 aa, synthetic construct
  REGION 1..116: note = a2DL1-DS11 VH
EVQLVQSGAEVKKPGSSVKVSCKASGGTFSSYAISWVRQAPGQGLEWMGGIIPIFGTANYAQKFQGRVTITADESTSTAYMELSSLRSEDTAVYYCARGLRFFDYWGQGTLVTVSS

SEQ ID NO: 128 - protein, 110 aa, synthetic construct
  REGION 1..110: note = a2DL1-DS11 VL
QSVLTQPPSASGTPGQRVTISCSGSSSNIGTNTVNWYQQFPGTAPKLLIYSNNQRPSGVPDRFSGSKSGTSGSLAISGLQSEDEADYYCAAWDDSLQGWLFGGGTKLTVL

SEQ ID NO: 129 - protein, 122 aa, synthetic construct
  REGION 1..122: note = a2DL1-DS12 VH
QVQLVQSGAEVKKPGSSVKVSCKASGGAFSSYAISWVRQAPGQGLEWMGGIIPIFGTANYAQKFQGRVTITADESTSTAYMELSSLRSEDTAVYYCARDPSSGWGYYGMDVWGQGTMVTVSS

SEQ ID NO: 130 - protein, 109 aa, synthetic construct
  REGION 1..109: note = a2DL1-DS12 VL
QSVVTQPPSVSGAPGQRVTISCTGDNSNLGAGYNVHWYQHLPGTAPKLLIYGNDNRPSGVPDRFSGSKSGTSASLAITGLQAEDEGDYYCQSYDSSLVVFGGGTKVTVL

SEQ ID NO: 131 - protein, 115 aa, synthetic construct
  REGION 1..115: note = a2DL1-DS13 VH
EVQLVQSGAEVKKPGSSVKVSCKASGGTFSSYAISWVRQAPGQGLEWMGGIIPIFGTANYAQKFQGRVTITADESTSTAYMELSSLRSEDTAVYYCARGFNPDYWGQGTLVTVSS

SEQ ID NO: 132 - protein, 110 aa, synthetic construct
  REGION 1..110: note = a2DL1-DS13 VL
QSVLTQPPSASGTPGQRVTISCSGSSSNIGSNTVNWYQQLPQTAPKLLIHHNNQRHSGVSDRFSASKSGTSASLAISGLQSEDEADYYCAAWDDTLTGLIFGGGTKLTVL

SEQ ID NO: 133 - protein, 125 aa, synthetic construct
  REGION 1..125: note = a2DL1-DS14 VH
QVQLQQSGPGLVKPSQTLSLTCAISGDSVSSNNAAWNWIRQSPSRGLEWLGRTYYRSKWYNDYAVSVKSRITINPDTSKNQFSLQLNSVTPEDTAVYYCARVPGDYYYYYGMDVWGQGTLVTVSS

SEQ ID NO: 134 - protein, 111 aa, synthetic construct
  REGION 1..111: note = a2DL1-DS14 VL
QSVLTQPPSVSGAPGQRVTISCTGSSSNIGAGYDVHWYQHLPGTAPKLLIYGNSNRPSGVPARFSGSKSGTSASLAITGLQAEDEADYYCQSYDIGLSGVVFGGGTKVTVL

SEQ ID NO: 135 - protein, 126 aa, synthetic construct
  REGION 1..126: note = a2DL1-DS15 VH
EVQLVQSGAEVKKPGSSVKVSCKASGGTFSSYAISWVRQAPGQGLEWMGGIIPIFGTANYAQKFQGRVTITADESTSTAYMELSSLRSEDTAVYYCAREELGYSSSSDYYYGMDVWGQGTLVTVSS

SEQ ID NO: 136 - protein, 112 aa, synthetic construct
  REGION 1..112: note = a2DL1-DS15 VL
QSVVTQPPSVSGAPGQRVTISCTGSSSNIGAGYDVHWYQQLPGTAPKLLIYGNSNRPSGVPDRFSGSKSGTSASLAVTGLQAEDEADYYCQSYDFRLGGFVIFGGGTKVTVL

SEQ ID NO: 137 - protein, 122 aa, synthetic construct
  REGION 1..122: note = a3DL1-DS2 VH
QVQLQQSGPGLVKPSQTLSLTCAISGDSVSSNSAAWNWIRQSPSRGLEWLGRTYYRSKWYNDYAVSVKSRITINPDTSKNQFSLQLNSMTPEDTAVYYCAREEGVSDAFDVWGQGTLVTVSS

SEQ ID NO: 138 - protein, 107 aa, synthetic construct
  REGION 1..107: note = a3DL1-DS2 VL
NIQMTQSPSSLSASVGDRVTITCRASQSISSYLNWYQQKPGKAPKLLIYAASSLQSGVPSRFSGSGSGTDFTLTISSLQPEDFATYYCQQSYSTPPTFGQGTKVEIK

SEQ ID NO: 139 - protein, 122 aa, synthetic construct
  REGION 1..122: note = a3DL1-DS3 VH
QVQLQQSGPGLVKPSQTLSLTCAISGDSVSSDSAAWNWIRQSPSRGLEWLGRTYYRSKWYNDYAVSVKSRITINPDTSKNQFSLQLNSVTPEDTAVYYCAREEGVSDAFDVWGQGTLVTVSS

SEQ ID NO: 140 - protein, 108 aa, synthetic construct
  REGION 1..108: note = a3DL1-DS3 VL
NIQMTQSPSSLSASVGDRVTITCRASQSISSYLNWYQQKPGKAPKLLIYAASSLQSGVPSRFSGSGSGTDFTLTISSLQPEDFATYYCQQSYSTPSLTFGGGTKVEIK

SEQ ID NO: 141 - protein, 126 aa, synthetic construct
  REGION 1..126: note = a3DL1-DS4 VH
EVQLVESGGGVVQPGRSLRLSCAASGFTFDDYAMHWVRQVPGKGLEWVAVISYDGSNKYYADSVKGRFTISRDNSKNTLYLQMNSLRAEDTAVYYCAREGTYGDSIHYYYYGMDVWGQGTMVTVSS

SEQ ID NO: 142 - protein, 108 aa, synthetic construct
  REGION 1..108: note = a3DL1-DS4 VL
EIVMTQSPATLSLSPGERATLSCRASQSVSSSYLSWYQQKPGQAPRLLMYGASTRATGIPARFSGSGSGTDFTLTISSLQPEDFAVYYCQQDYNLPLTFGGGTKLEIK

SEQ ID NO: 143 - protein, 122 aa, synthetic construct
  REGION 1..122: note = a3DL1-DS5 VH
QVQLQQSGPGLVKPSQTLSLTCAISGDSVSSNSAAWNWIRQSPSRGLEWLGRTYYRSKWYNDYAVSVKSRITINPDTSKNQFSLQLNSVTPEDTAVYYCAREMGWYDWFDPWGQGTLVTVSS

SEQ ID NO: 144 - protein, 107 aa, synthetic construct
  REGION 1..107: note = a3DL1-DS5 VL
DIQMTQSPSSLSASVGDRVTITCRASQSISTYLNWYQQKPGKAPKLLIYAASSLQSGVPSRFSGSGSGTDFTLTISSLQPEDFATYYCQQSYSTPITFGQGTRLEIK

SEQ ID NO: 145 - protein, 120 aa, synthetic construct
  REGION 1..120: note = a3DL1-DS6 VH
QMQLVQSGAEVKKPGESLKISCKGSGYSFTSYWIGWVRQMPGKGPEWMGIIYPGDSYTNYSPSFQGHVTISADKSISTAYLQWSSLKASDTAMYYCARLAPTVEDAFDIWGQGTLVTVSS

SEQ ID NO: 146 - protein, 111 aa, synthetic construct
  REGION 1..111: note = a3DL1-DS6 VL
QSVLTQPPSVSEAPGQRVTISCTGSSSNIGAGYDVHWYQQLPGTAPKLLIYGNSNRPSGVPDRFSGSKSGTSASLAITGLQAEDEADYYCQSYDSSLSEEVFGTGTKVTVL